European Patent Application EP 4 410 953 A1, published August 7, 2024. Title: Novel probiotics and use thereof. Applicant: 피비엘바이오랩 주식회사. The sequence listing filed with the application follows.

SEQUENCE LISTING (11 sequences)

SEQ ID NO: 1 - DNA, 1395 bp, synthetic construct
  misc_feature 1..1395: note = Lactobacillus rhamnosus NK210
  source 1..1395: mol_type = other DNA
ctgcccttaagtgggggataacatttggaaacagatgctaataccgcataaatccaagaaccgcatggttcttggctgaaagatggcgtaagctatcgcttttggatggacccgcggcgtattagctagttggtgaggtaacggctcaccaaggcaatgatacgtagccgaactgagaggttgatcggccacattgggactgagacacggcccaaactcctacgggaggcagcagtagggaatcttccacaatggacgcaagtctgatggagcaacgccgcgtgagtgaagaaggctttcgggtcgtaaaactctgttgttggagaagaatggtcggcagagtaactgttgtcggcgtgacggtatccaaccagaaagccacggctaactacgtgccagcagccgcggtaatacgtaggtggcaagcgttatccggatttattgggcgtaaagcgagcgcaggcggttttttaagtctgatgtgaaagccctcggcttaaccgaggaagtgcatcggaaactggraaacttgagtgcagaagaggacagtggaactccatgtgtagcggtgaaatgcgtagatatatggaagaacaccagtggcgaaggcggctgtctggtctgtaactgacgctgaggctcgaaagcatgggtagcgaacaggattagataccctggtagtccatgccgtaaacgatgaatgctaggtgttggagggtttccgcccttcagtgccgcagctaacgcattaagcattccgcctggggagtacgaccgcaaggttgaaactcaaaggaattgacgggggcccgcacaagcggtggagcatgtggtttaattcgaagcaacgcgaagaaccttaccaggtcttgacatcttttgatcacctgagagatcaggtttccccttcgggggcaaaatgacaggtggtgcatggttgtcgtcagctcgtgtcgtgagatgttgggttaagtcccgcaacgagcgcaacccttatgactagttgccagcatttagttgggcactctagtaagactgccggtgacaaaccggaggaaggtggggatgacgtcaaatcatcatgccccttatgacctgggctacacacgtgctacaatggatggtacaacgagttgcgagaccgcgaggtcaagctaatctcttaaagccattctcagttcggactgtaggctgcaactcgcctacacgaagtcggaatcgctagtaatcgcggatcagcacgccgcggtgaatacgttcccgggccttgtacacaccgcccgtcacaccatgagagtttgtaacacccgaagccggtggcgtaacccttttagggagcgagccgtctaaggtgggacaaatgattagggtgaagtcgtaacagaggtaaccgta

SEQ ID NO: 2 - DNA, 1461 bp, synthetic construct
  misc_feature 1..1461: note = Bifidobacterium longum NK219
  source 1..1461: mol_type = other DNA
ctcaggatgaacgctggcggcgtgcttaacacatgcaagtcgaacgggatccatcaggctttgcttggtggtgagagtggcgaacgggtgagtaatgcgtgaccgacctgccccatacaccggaatagctcctggaaacgggtggtaatgccggatgctccagttgatcgcatggtcttctgggaaagctttcgcggtatgggatggggtcgcgtcctatcagcttgacggcggggtaacggcccaccgtggcttcgacgggtagccggcctgagagggcgaccggccacattgggactgagatacggcccagactcctacgggaggcagcagtggggaatattgcacaatgggcgcaagcctgatgcagcgacgccgcgtgagggatggaggccttcgggttgtaaacctcttttatcggggagcaagcgagagtgagtttacccgttgaataagcaccggctaactacgtgccagcagccgcggtaatacgtagggtgcaagcgttatccggaattattgggcgtaaagggctcgtaggcggttcgtcgcgtccggtgtgaaagtccatcgcttaacggtggatccgcgccgggtacgggcgggcttgagtgcggtaggggagactggaattcccggtgtaacggtggaatgtgtagatatcgggaagaacaccaatggcgaaggcaggtctctgggccgttactgacgctgaggagcgaaagcgtggggagcgaacaggattagataccctggtagtccacgccgtaaacggtggatgctggatgtggggcccgttccacgggttccgtgtcggagctaacgcgttaagcatcccgcctggggagtacggccgcaaggctaaaactcaaagaaattgacgggggcccgcacaagcggcggagcatgcggattaattcgatgcaacgcgaagaaccttacctgggcttgacatgttcccgacggtcgtagagatacggcttcccttcggggcgggttcacaggtggtgcatggtcgtcgtcagctcgtgtcgtgagatgttgggttaagtcccgcaacgagcgcaaccctcgccccgtgttgccagcggattatgccgggaactcacgggggaccgccggggttaactcggaggaaggtggggatgacgtcagatcatcatgccccttacgtccagggcttcacgcatgctacaatggccggtacaacgggatgcgacgcggcgacgcggagcggatccctgaaaaccggtctcagttcggatcgcagtctgcaactcgactgcgtgaaggcggagtcgctagtaatcgcgaatcagcaacgtcgcggtgaatgcgttcccgggccttgtacacaccgcccgtcaagtcatgaaagtgggcagcacccgaagccggtggcctaacctcttgtgggatggagccgtctaaggtgaggctcgtgattgggactaagtcgta

SEQ ID NO: 3 - DNA, 1361 bp, synthetic construct
  misc_feature 1..1361: note = Lactococcus lactis NK209
  source 1..1361: mol_type = other DNA
ggggacaacatttggaaacgaatgctaataccgcataaaaactttaaacacaagttttaagtttgaaagatgcaattgcatcactcaaagatgatcccgcgttgtattagctagttggtgaggtaaaggctcaccaaggcgatgatacatagccgacctgagagggtgatcggccacattgggactgagacacggcccaaactcctacgggaggcagcagtagggaatcttcggcaatggacgaaagtctgaccgagcaacgccgcgtgagtgaagaaggttttcggatcgtaaaactctgttggtagagaagaacgttggtgagagtggaaagctcatcaagtgacggtaactacccagaaagggacggctaactacgtgccagcagccgcggtaatacgtaggtcccgagcgttgtccggatttattgggcgtaaagcgagcgcaggtggtttattaagtctggtgtaaaaggcagtggctcaaccattgtatgcattggaaactggtagacttgagtgcaggagaggagagtggaattccatgtgtagcggtgaaatgcgtagatatatggaggaacaccggtggcgaaagcggctctctggcctgtaactgacactgaggctcgaaagcgtggggagcaaacaggattagataccctggtagtccacgccgtaaacgatgagtgctagatgtagggagctataagttctctgtatcgcagctaacgcaataagcactccgcctggggagtacgaccgcaaggttgaaactcaaaggaattgacgggggcccgcacaagcggtggagcatgtggtttaattcgaagcaacgcgaagaaccttaccaggtcttgacatactcgtgctattcctagagataggaagttccttcgggacacgggatacaggtggtgcatggttgtcgtcagctcgtgtcgtgagatgttgggttaagtcccgcaacgagcgcaacccctattgttagttgccatcattaagttgggcactctaacgagactgccggtgataaaccggaggaaggtggggatgacgtcaaatcatcatgccccttatgacctgggctacacacgtgctacaatggatggtacaacgagtcgcgagacagtgatgtttagctaatctcttaaaaccattctcagttcggattgtaggctgcaactcgcctacatgaagtcggaatcgctagtaatcgcggatcagcacgccgcggtgaatacgttcccgggccttgtacacaccgcccgtcacaccacgggagttgggagtacccgaagtaggttgcctaaccgcaaggagggcgcttcctaaggtaagaccgatgactggggtgaagtcgta

SEQ ID NO: 4 - DNA, 21 bp, synthetic construct
  misc_feature 1..21: note = Clostridium difficile forward primer
  source 1..21: mol_type = other DNA
gggagcttcccatacgggttg

SEQ ID NO: 5 - DNA, 22 bp, synthetic construct
  misc_feature 1..22: note = Clostridium difficile reverse primer
  source 1..22: mol_type = other DNA
ttgactgcctcaatgcttgggc

SEQ ID NO: 6 - DNA, 20 bp, synthetic construct
  misc_feature 1..20: note = Foxp3 forward primer
  source 1..20: mol_type = other DNA
agaagctgggagctatgcag

SEQ ID NO: 7 - DNA, 19 bp, synthetic construct
  misc_feature 1..19: note = Foxp3 reverse primer
  source 1..19: mol_type = other DNA
gctacgatgcagcaagcgc

SEQ ID NO: 8 - DNA, 22 bp, synthetic construct
  misc_feature 1..22: note = Tbet forward primer
  source 1..22: mol_type = other DNA
tgcccgaactacagtcacgaac

SEQ ID NO: 9 - DNA, 22 bp, synthetic construct
  misc_feature 1..22: note = Tbet reverse primer
  source 1..22: mol_type = other DNA
agtgacctcgcctggtgaaatg

SEQ ID NO: 10 - DNA, 20 bp, synthetic construct
  misc_feature 1..20: note = GAPDH forward primer
  source 1..20: mol_type = other DNA
tgcagtggcaaagtggagat

SEQ ID NO: 11 - DNA, 21 bp, synthetic construct
  misc_feature 1..21: note = GAPDH reverse primer
  source 1..21: mol_type = other DNA
tttgccgtgagtggagtcata